European Patent Specification EP 3 483 311 B1, published September 17, 2025. Title: METHODS FOR NUCLEIC ACID ASSEMBLY AND HIGH THROUGHPUT SEQUENCING. Applicant: Gen9, Inc. Application EP. The sequence listing filed with the application follows.

SEQUENCE LISTING (1 sequence)

SEQ ID NO: 1 - DNA, 2608 bp, Artificial Sequence
  Synthetic Construct
tcgcgcgtttcggtgatgacggtgaaaacctctgacacatgcagctcccggagacggtcacagcttgtctgtaagcggatgccgggagcagacaagcccgtcagggcgcgtcagcgggtgttggcgggtgtcggggctggcttaactatgcggcatcagagcagattgtactgagagtgcaccatatgcggtgtgaaataccgcacagatgcgtaaggagaaaataccgcatcaggcgccattcgccattcaggctgcgcaactgttgggaagggcgatcggtgcgggcctcttcgctattacgccagctggcgaaagggggatgtgctgcaaggcgattaagttgggtaacgccagggttttcccagtcacgacgttgtaaaacgacggccagtgaattagtgttgagaccattcagctccggtctcgacactgagcttggcgtaatcatggtcatagctgtttcctgtgtgaaattgttatccgctcacaattccacacaacatacgagccggaagcataaagtgtaaagcctggggtgcctaatgagtgagctaactcacattaattgcgttgcgctcactgcccgctttccagtcgggaaacctgtcgtgccagctgcattaatgaatcggccaacgcgcggggagaggcggtttgcgtattgggcgctcttccgcttcctcgctcactgactcgctgcgctcggtcgttcggctgcggcgagcggtatcagctcactcaaaggcggtaatacggttatccacagaatcaggggataacgcaggaaagaacatgtgagcaaaaggccagcaaaaggccaggaaccgtaaaaaggccgcgttgctggcgtttttccataggctccgcccccctgacgagcatcacaaaaatcgacgctcaagtcagaggtggcgaaacccgacaggactataaagataccaggcgtttccccctggaagctccctcgtgcgctctcctgttccgaccctgccgcttaccggatacctgtccgcctttctcccttcgggaagcgtggcgctttctcatagctcacgctgtaggtatctcagttcggtgtaggtcgttcgctccaagctgggctgtgtgcacgaaccccccgttcagcccgaccgctgcgccttatccggtaactatcgtcttgagtccaacccggtaagacacgacttatcgccactggcagcagccactggtaacaggattagcagagcgaggtatgtaggcggtgctacagagttcttgaagtggtggcctaactacggctacactagaagaacagtatttggtatctgcgctctgctgaagccagttaccttcggaaaaagagttggtagctcttgatccggcaaacaaaccaccgctggtagcggtggtttttttgtttgcaagcagcagattacgcgcagaaaaaaaggatctcaagaagatcctttgatcttttctacggggtctgacgctcagtggaacgaaaactcacgttaagggattttggtcatgagattatcaaaaaggatcttcacctagatccttttaaattaaaaatgaagttttaaatcaatctaaagtatatatgagtaaacttggtctgacagtcagaagaactcgtcaagaaggcgatagaaggcgatgcgctgcgaatcgggagcggcgataccgtaaagcacgaggaagcggtcagcccattcgccgccaagctcttcagcaatatcacgggtagccaacgctatgtcctgatagcggtccgccacacccagccggccacagtcgatgaatccagaaaagcggccattttccaccatgatattcggcaagcaggcatcgccatgggtcacgacgagatcctcgccgtcgggcatgctcgccttgagcctggcgaacagttcggctggcgcgagcccctgatgctcttcgtccagatcatcctgatcgacaagaccggcttccatccgagtacgtgctcgctcgatgcgatgtttcgcttggtggtcgaatgggcaggtagccggatcaagcgtatgcagccgccgcattgcatcagccatgatggatactttctcggcaggagcaaggtgagatgacaggagatcctgccccggcacttcgcccaatagcagccagtcccttcccgcttcagtgacaacgtcgagcacagctgcgcaaggaacgcccgtcgtggccagccacgatagccgcgctgcctcgtcttgcagttcattcagggcaccggacaggtcggtcttgacaaaaagaaccgggcgcccctgcgctgacagccggaacacggcggcatcagagcagccgattgtctgttgtgcccagtcatagccgaatagcctctccacccaagcggccggagaacctgcgtgcaatccatcttgttcaatcatactcttcctttttcaatattattgaagcatttatcagggttattgtctcatgagcggatacatatttgaatgtatttagaaaaataaacaaataggggttccgcgcacatttccccgaaaagtgccacctgacgtctaagaaaccattattatcatgacattaacctataaaaataggcgtatcacgaggccctttcgtc